European Patent Specification EP 3 182 979 B1, published December 6, 2023. Title: Novel Compositions and Methods Useful For Treating or Preventing Liver Diseases or Disorders, and Promoting Weight Loss. Applicant: Yale University Mehal, Wajahat Ouyang, Xinshou. The sequence listing filed with the application follows.

SEQUENCE LISTING (12 sequences)

SEQ ID NO: 1 - DNA, 18 bp, Artificial Sequence
  chemically synthesized
aaatggcctccctctcat

SEQ ID NO: 2 - DNA, 18 bp, Artificial Sequence
  chemically synthesized
cctccacttggtggtttg

SEQ ID NO: 3 - DNA, 20 bp, Artificial Sequence
  chemically synthesized
tgcaggaggaagactttgtg

SEQ ID NO: 4 - DNA, 20 bp, Artificial Sequence
  chemically synthesized
cacgtggtccattctggtag

SEQ ID NO: 5 - DNA, 18 bp, Artificial Sequence
  chemically synthesized
ccaggccttgacaagcta

SEQ ID NO: 6 - DNA, 18 bp, Artificial Sequence
  chemically synthesized
cgcggagaaagagacaag

SEQ ID NO: 7 - DNA, 20 bp, Artificial Sequence
  chemically synthesized
tgcaagagacttccatccag

SEQ ID NO: 8 - DNA, 20 bp, Artificial Sequence
  chemically synthesized
tgaagtctcctctccggact

SEQ ID NO: 9 - DNA, 19 bp, Artificial Sequence
  chemically synthesized
caagagcctcagagtgcag

SEQ ID NO: 10 - DNA, 19 bp, Artificial Sequence
  chemically synthesized
ccagggacactgacgtaga

SEQ ID NO: 11 - DNA, 20 bp, Artificial Sequence
  chemically synthesized
agtaaggcctgtagctgtgc

SEQ ID NO: 12 - DNA, 20 bp, Artificial Sequence
  chemically synthesized
cgctggtataaggtggtctc